European Patent Specification EP 3 626 747 B1, published July 19, 2023. Title: NOVEL RECOMBINANT BI-FUNCTIONAL FUSION PROTEIN, PREPARATION METHOD THEREFOR AND USE THEREOF. Applicant: ImmuneOnco Biopharmaceuticals (Shanghai) Co., Ltd. Application PCT/CN2018/079187. The sequence listing filed with the application follows.

SEQUENCE LISTING (13 sequences)

SEQ ID NO: 1 - DNA, 1752 bp, Artificial Sequence
  heavy chain-SD1
caggtccagctgcagcagccgggcgcggagctcgtgaagccgggggcctcggtcaagatgagctgcaaggccagcggctacaccttcacgagctacaacatgcactgggtgaagcagaccccgggccgggggctggagtggatcggcgccatctaccccgggaacggcgacaccagctacaaccagaagttcaagggcaaggcgaccctgacggcggacaagtcgagcagcaccgcctacatgcagctcagcagcctgacctcggaggacagcgccgtctactactgcgcccggtccacgtactacggcggcgactggtacttcaacgtctggggggccggcacgaccgtgaccgtgagcgcggctagcaccaagggcccatcggtcttccccctggcaccctcctccaagagcacctctgggggcacagcggccctgggctgcctggtcaaggactacttccccgaaccggtgacggtgtcgtggaactcaggcgccctgaccagcggcgtgcacaccttcccggctgtcctacagtcctcaggactctactccctcagcagcgtggtgaccgtgccctccagcagcttgggcacccagacctacatctgcaacgtgaatcacaagcccagcaacaccaaggtggacaagagagttgagcccaaatcttgtgacaaaactcacacatgcccaccgtgcccagcacctgaactcctggggggaccgtcagtcttcctcttccccccaaaacccaaggacaccctcatgatctcccggacccctgaggtcacatgcgtggtggtggacgtgagccacgaagaccctgaggtcaagttcaactggtatgtggacggcgtggaggtgcataatgccaagacaaagccgcgggaggagcagtacaacgccacgtaccgtgtggtcagcgtcctcaccgtcctgcaccaagactggctgaatggcaaggagtacaagtgcaaggtctccaacaaagccctcccagcccccatcgccgcaaccatctccaaagccaaagggcagccccgagaaccacaggtgtacaccctgcccccatcccgggaggagatgaccaagaaccaagtcagcctgacctgcctggtcaaaggcttctatcccagcgacatcgccgtggagtgggagagcaatgggcagccggagaacaactacaagaccacgcctcccgtgctggactccgacggctccttcttcctctattccaagctcaccgtggacaagagcaggtggcagcaggggaacgtcttctcatgctccgtgatgcatgaggctctgcacaaccactacacgcagaagagcctctccctgtctccgggcgaggaggagctgcaggtgattcagcctgacaagtccgtatcagttgcagctggagagtcggccattctgcactgcactgtgacctccctgatccctgtggggcccatccagtggttcagaggagctggaccagcccgggaattaatctacaatcaaaaagaaggccacttcccccgggtaacaactgtttcagagtccacaaagagagaaaacatggacttttccatcagcatcagtgccatcaccccagcagatgccggcacctactactgtgtgaagttccggaaagggagccctgacacggagtttaagtctggagcaggcactgagctgtctgtgcgtgccaaaccctctgcccccgtggtatcgggccctgcggcgagggccacacctcagcactga

SEQ ID NO: 2 - DNA, 642 bp, Artificial Sequence
  light chain
cagatcgtgctgagccagtcgccggccatcctcagcgcgagccccggcgagaaggtcaccatgacgtgccgggccagcagctcggtgagctacatccactggttccagcagaagcccgggagcagccccaagccgtggatctacgccaccagcaacctggcctcgggcgtgcccgtgcgcttcagcgggagcggcagcgggaccagctacagcctgaccatctcgcgggtcgaggccgaggacgccgccacctactactgccagcagtggacctccaacccgcccacgttcggcggcggcaccaagcacgagctgaagcgaactgtggctgcaccatctgtcttcatcttcccgccatctgatgagcagttgaaatctggaactgcctctgttgtgtgcctgctgaataacttctatcccagagaggccaaagtacagtggaaggtggataacgccctccaatcgggtaactcccaggagagtgtcacagagcaggacagcaaggacagcacctacagcctcagcagcaccctgacgctgagcaaagcagactacgagaaacacaaagtctacgcctgcgaagtcacccatcagggcctgagctcgcccgtcacaaagagcttcaacaggggagagtgttag

SEQ ID NO: 3 - protein, 583 aa, Artificial Sequence
  heavy chain-SD1
QVQLQQPGAELVKPGASVKMSCKASGYTFTSYNMHWVKQTPGRGLEWIGAIYPGNGDTSYNQKFKGKATLTADKSSSTAYMQLSSLTSEDSAVYYCARSTYYGGDWYFNVWGAGTTVTVSAASTKGPSVFPLAPSSKSTSGGTAALGCLVKDYFPEPVTVSWNSGALTSGVHTFPAVLQSSGLYSLSSVVTVPSSSLGTQTYICNVNHKPSNTKVDKRVEPKSCDKTHTCPPCPAPELLGGPSVFLFPPKPKDTLMISRTPEVTCVVVDVSHEDPEVKFNWYVDGVEVHNAKTKPREEQYNATYRVVSVLTVLHQDWLNGKEYKCKVSNKALPAPIAATISKAKGQPREPQVYTLPPSREEMTKNQVSLTCLVKGFYPSDIAVEWESNGQPENNYKTTPPVLDSDGSFFLYSKLTVDKSRWQQGNVFSCSVMHEALHNHYTQKSLSLSPGEEELQVIQPDKSVSVAAGESAILHCTVTSLIPVGPIQWFRGAGPARELIYNQKEGHFPRVTTVSESTKRENMDFSISISAITPADAGTYYCVKFRKGSPDTEFKSGAGTELSVRAKPSAPVVSGPAARATPQH

SEQ ID NO: 4 - protein, 213 aa, Artificial Sequence
  light chain
QIVLSQSPAILSASPGEKVTMTCRASSSVSYIHWFQQKPGSSPKPWIYATSNLASGVPVRFSGSGSGTSYSLTISRVEAEDAATYYCQQWTSNPPTFGGGTKHELKRTVAAPSVFIFPPSDEQLKSGTASVVCLLNNFYPREAKVQWKVDNALQSGNSQESVTEQDSKDSTYSLSSTLTLSKADYEKHKVYACEVTHQGLSSPVTKSFNRGEC

SEQ ID NO: 5 - protein, 121 aa, Artificial Sequence [sequence omitted]

SEQ ID NO: 6 - DNA, 363 bp, Artificial Sequence
  VH
caggtccagctgcagcagccgggcgcggagctcgtgaagccgggggcctcggtcaagatgagctgcaaggccagcggctacaccttcacgagctacaacatgcactgggtgaagcagaccccgggccgggggctggagtggatcggcgccatctaccccgggaacggcgacaccagctacaaccagaagttcaagggcaaggcgaccctgacggcggacaagtcgagcagcaccgcctacatgcagctcagcagcctgacctcggaggacagcgccgtctactactgcgcccggtccacgtactacggcggcgactggtacttcaacgtctggggggccggcacgaccgtgaccgtgagcgcg

SEQ ID NO: 7 - protein, 106 aa, Artificial Sequence [sequence omitted]

SEQ ID NO: 8 - DNA, 318 bp, Artificial Sequence
  VL
cagatcgtgctgagccagtcgccggccatcctcagcgcgagccccggcgagaaggtcaccatgacgtgccgggccagcagctcggtgagctacatccactggttccagcagaagcccgggagcagccccaagccgtggatctacgccaccagcaacctggcctcgggcgtgcccgtgcgcttcagcgggagcggcagcgggaccagctacagcctgaccatctcgcgggtcgaggccgaggacgccgccacctactactgccagcagtggacctccaacccgcccacgttcggcggcggcaccaagctcgagatcaag

SEQ ID NO: 9 - protein, 133 aa, Artificial Sequence
  SD1
EEELQVIQPDKSVSVAAGESAILHCTVTSLIPVGPIQWFRGAGPARELIYNQKEGHFPRVTTVSESTKRENMDFSISISAITPADAGTYYCVKFRKGSPDTEFKSGAGTELSVRAKPSAPVVSGPAARATPQH

SEQ ID NO: 10 - protein, 213 aa, Artificial Sequence; identical to SEQ ID NO: 4
  light chain

SEQ ID NO: 11 - DNA, 1785 bp, Artificial Sequence
  SD1-heavy chain
gaggaggagctgcaggtgattcagcctgacaagtccgtatcagttgcagctggagagtcggccattctgcactgcactgtgacctccctgatccctgtggggcccatccagtggttcagaggagctggaccagcccgggaattaatctacaatcaaaaagaaggccacttcccccgggtaacaactgtttcagagtccacaaagagagaaaacatggacttttccatcagcatcagtgccatcaccccagcagatgccggcacctactactgtgtgaagttccggaaagggagccctgacacggagtttaagtctggagcaggcactgagctgtctgtgcgtgccaaaccctctgcccccgtggtatcgggccctgcggcgagggccacacctcagcacggcggcggtgggagcggcggcgggggctcgcaggtccagctgcagcagccgggcgcggagctcgtgaagccgggggcctcggtcaagatgagctgcaaggccagcggctacaccttcacgagctacaacatgcactgggtgaagcagaccccgggccgggggctggagtggatcggcgccatctaccccgggaacggcgacaccagctacaaccagaagttcaagggcaaggcgaccctgacggcggacaagtcgagcagcaccgcctacatgcagctcagcagcctgacctcggaggacagcgccgtctactactgcgcccggtccacgtactacggcggcgactggtacttcaacgtctggggggccggcacgaccgtgaccgtgagcgcggctagcaccaagggcccatcggtcttccccctggcaccctcctccaagagcacctctgggggcacagcggccctgggctgcctggtcaaggactacttccccgaaccggtgacggtgtcgtggaactcaggcgccctgaccagcggcgtgcacaccttcccggctgtcctacagtcctcaggactctactccctcagcagcgtggtgaccgtgccctccagcagcttgggcacccagacctacatctgcaacgtgaatcacaagcccagcaacaccaaggtggacaagagagttgagcccaaatcttgtgacaaaactcacacatgcccaccgtgcccagcacctgaactcctggggggaccgtcagtcttcctcttccccccaaaacccaaggacaccctcatgatctcccggacccctgaggtcacatgcgtggtggtggacgtgagccacgaagaccctgaggtcaagttcaactggtatgtggacggcgtggaggtgcataatgccaagacaaagccgcgggaggagcagtacaacgccacgtaccgtgtggtcagcgtcctcaccgtcctgcaccaagactggctgaatggcaaggagtacaagtgcaaggtctccaacaaagccctcccagcccccatcgccgcaaccatctccaaagccaaagggcagccccgagaaccacaggtgtacaccctgcccccatcccgggaggagatgaccaagaaccaagtcagcctgacctgcctggtcaaaggcttctatcccagcgacatcgccgtggagtgggagagcaatgggcagccggagaacaactacaagaccacgcctcccgtgctggactccgacggctccttcttcctctattccaagctcaccgtggacaagagcaggtggcagcaggggaacgtcttctcatgctccgtgatgcatgaggctctgcacaaccactacacgcagaagagcctctccctgtctccgggcaaatga

SEQ ID NO: 12 - DNA, 642 bp, Artificial Sequence; identical to SEQ ID NO: 2
  light chain

SEQ ID NO: 13 - protein, 594 aa, Artificial Sequence
  SD1-heavy chain
EEELQVIQPDKSVSVAAGESAILHCTVTSLIPVGPIQWFRGAGPARELIYNQKEGHFPRVTTVSESTKRENMDFSISISAITPADAGTYYCVKFRKGSPDTEFKSGAGTELSVRAKPSAPVVSGPAARATPQHGGGGSGGGGSQVQLQQPGAELVKPGASVKMSCKASGYTFTSYNMHWVKQTPGRGLEWIGAIYPGNGDTSYNQKFKGKATLTADKSSSTAYMQLSSLTSEDSAVYYCARSTYYGGDWYFNVWGAGTTVTVSAASTKGPSVFPLAPSSKSTSGGTAALGCLVKDYFPEPVTVSWNSGALTSGVHTFPAVLQSSGLYSLSSVVTVPSSSLGTQTYICNVNHKPSNTKVDKRVEPKSCDKTHTCPPCPAPELLGGPSVFLFPPKPKDTLMISRTPEVTCVVVDVSHEDPEVKFNWYVDGVEVHNAKTKPREEQYNATYRVVSVLTVLHQDWLNGKEYKCKVSNKALPAPIAATISKAKGQPREPQVYTLPPSREEMTKNQVSLTCLVKGFYPSDIAVEWESNGQPENNYKTTPPVLDSDGSFFLYSKLTVDKSRWQQGNVFSCSVMHEALHNHYTQKSLSLSPGK